European Patent Specification EP 3 611 179 B1, published March 1, 2023. Title: Novel steviol glycoside and production method for same, and sweetener composition containing same. Applicant: SUNTORY HOLDINGS LIMITED. The sequence listing filed with the application follows.

SEQUENCE LISTING (36 sequences)

SEQ ID NO: 1 - DNA, 1446 bp, Stevia rebaudiana
  CDS (1)..(1446)
atggatgcaatggctacaactgagaagaaaccacacgtcatcttcataccatttccagcacaaagccacattaaagccatgctcaaactagcacaacttctccaccacaaaggactccagataaccttcgtcaacaccgacttcatccacaaccagtttcttgaatcatcgggcccacattgtttggacggttcaccgggtttccggttcgaaaccatcccggatggtgtttctcacagtccggaagcgagcatcccaatcagagaatcactcttgagatccattgaaaccaacttcttggatcgtttcattgatcttgtaaccaaacttccggatcctccgacttgtattatctcagatgggttcttgtcggttttcacaattgacgctgcaaaaaagcttggaattccggtcatgatgtattggacacttgctgcctgtgggttcatgggtttttaccatattcattctctcattgagaaaggatttgcaccacttaaagatgcaagttacttgacaaatgggtatttggacaccgtcattgattgggttccgggaatggaaggcatccgtctcaaggatttcccgctggactggagcactgacctcaatgacaaagttttgatgttcactacagaagctcctcaaaggtcacacaaggtttcacatcatattttccacacgttcgatgagttggagcctagtattataaaaactttgtcattgaggtataatcacatttacaccatcggcccactgcaattacttcttgatcaaatacccgaagagaaaaagcaaactggaattacgagtctccatggatacagtttagtaaaagaagaaccagagtgtttccagtggcttcagtctaaagaaccaaattccgtcgtttatgtaaattttggaagtactacagtaatgtctttagaagacatgacggaatttggttggggacttgctaatagcaaccattatttcctttggatcatccgatcaaacttggtgataggggaaaatgcagttttgccccctgaacttgaggaacatataaagaaaagaggctttattgctagctggtgttcacaagaaaaggtcttgaagcacccttcggttggagggttcttgactcattgtgggtggggatcgaccatcgagagcttgtctgctggggtgccaatgatatgctggccttattcgtgggaccagctgaccaactgtaggtatatatgcaaagaatgggaggttgggctcgagatgggaaccaaagtgaaacgagatgaagtcaagaggcttgtacaagagttgatgggagaaggaggtcacaaaatgaggaacaaggctaaagattggaaagaaaaggctcgcattgcaatagctcctaacggttcatcttctttgaacatagacaaaatggtcaaggaaatcaccgtgctagcaagaaactag

SEQ ID NO: 2 - protein, 481 aa, Stevia rebaudiana
MDAMATTEKKPHVIFIPFPAQSHIKAMLKLAQLLHHKGLQITFVNTDFIHNQFLESSGPHCLDGSPGFRFETIPDGVSHSPEASIPIRESLLRSIETNFLDRFIDLVTKLPDPPTCIISDGFLSVFTIDAAKKLGIPVMMYWTLAACGFMGFYHIHSLIEKGFAPLKDASYLTNGYLDTVIDWVPGMEGIRLKDFPLDWSTDLNDKVLMFTTEAPQRSHKVSHHIFHTFDELEPSIIKTLSLRYNHIYTIGPLQLLLDQIPEEKKQTGITSLHGYSLVKEEPECFQWLQSKEPNSVVYVNFGSTTVMSLEDMTEFGWGLANSNHYFLWIIRSNLVIGENAVLPPELEEHIKKRGFIASWCSQEKVLKHPSVGGFLTHCGWGSTIESLSAGVPMICWPYSWDQLTNCRYICKEWEVGLEMGTKVKRDEVKRLVQELMGEGGHKMRNKAKDWKEKARIAIAPNGSSSLNIDKMVKEITVLARN

SEQ ID NO: 3 - DNA, 1383 bp, Stevia rebaudiana
  CDS (1)..(1383)
atggcggaacaacaaaagatcaagaaatcaccacacgttctactcatcccattccctttacaaggccatataaaccctttcatccagtttggcaaacgattaatctccaaaggtgtcaaaacaacacttgttaccaccatccacaccttaaactcaaccctaaaccacagtaacaccaccaccacctccatcgaaatccaagcaatttccgatggttgtgatgaaggcggttttatgagtgcaggagaatcatatttggaaacattcaaacaagttgggtctaaatcactagctgacttaatcaagaagcttcaaagtgaaggaaccacaattgatgcaatcatttatgattctatgactgaatgggttttagatgttgcaattgagtttggaatcgatggtggttcgtttttcactcaagcttgtgttgtaaacagcttatattatcatgttcataagggtttgatttctttgccattgggtgaaactgtttcggttcctggatttccagagcttcaacggtgggagacaccgttaattttgcagaatcatgagcaaatacagagcccttggtctcagatgttgtttggtcagtttgctaatattgatcaagcacgttgggtcttcacaaatagtttttacaagctcgaggaagaggtaatagagtggacgagaaagatatggaacttgaaggtaatcgggccaacacttccatccatgtaccttgacaaacgacttgatgatgataaagataacggatttaatctctacaaagcaaaccatcatgagtgcatgaactggttagacgataagccaaaggaatcagttgtttacgtagcatttggtagcctggtgaaacatggacccgaacaagtggaagaaatcacacgggctttaatagatagtgatgtcaacttcttgtgggttatcaaacataaagaagagggaaagctcccagaaaatctttcggaagtaataaaaaccggaaagggtttgattgtagcatggtgcaaacaattggatgtgttagcacacgaatcagtaggatgctttgttacacattgtgggttcaactcaactcttgaagcaataagtcttggagtccccgttgttgcaatgcctcaattttcggatcaaactacaaatgccaagcttctagatgaaattttgggtgttggagttagagttaaggctgatgagaatgggatagtgagaagaggaaatcttgcgtcatgtattaagatgattatggaggaggaaagaggagtaataatccgaaagaatgcggtaaaatggaaggatttggctaaagtagccgttcatgaaggtggtagctcagacaatgatattgtcgaatttgtaagtgagctaattaaggcttaa

SEQ ID NO: 4 - protein, 460 aa, Stevia rebaudiana
MAEQQKIKKSPHVLLIPFPLQGHINPFIQFGKRLISKGVKTTLVTTIHTLNSTLNHSNTTTTSIEIQAISDGCDEGGFMSAGESYLETFKQVGSKSLADLIKKLQSEGTTIDAIIYDSMTEWVLDVAIEFGIDGGSFFTQACVVNSLYYHVHKGLISLPLGETVSVPGFPELQRWETPLILQNHEQIQSPWSQMLFGQFANIDQARWVFTNSFYKLEEEVIEWTRKIWNLKVIGPTLPSMYLDKRLDDDKDNGFNLYKANHHECMNWLDDKPKESVVYVAFGSLVKHGPEQVEEITRALIDSDVNFLWVIKHKEEGKLPENLSEVIKTGKGLIVAWCKQLDVLAHESVGCFVTHCGFNSTLEAISLGVPVVAMPQFSDQTTNAKLLDEILGVGVRVKADENGIVRRGNLASCIKMIMEEERGVIIRKNAVKWKDLAKVAVHEGGSSDNDIVEFVSELIKA

SEQ ID NO: 5 - DNA, 1458 bp, Stevia rebaudiana
  CDS (1)..(1458)
atgtacaacgttacttatcatcaaaattcaaaagcaatggctaccagtgactccatagttgacgaccgtaagcagcttcatgttgcgacgttcccatggcttgctttcggtcacatcctcccttaccttcagctttcgaaattgatagctgaaaagggtcacaaagtctcgtttctttctaccaccagaaacattcaacgtctctcttctcatatctcgccactcataaatgttgttcaactcacacttccacgtgtccaagagctgccggaggatgcagaggcgaccactgacgtccaccctgaagatattccatatctcaagaaggcttctgatggtcttcaaccggaggtcacccggtttctagaacaacactctccggactggattatttatgattatactcactactggttgccatccatcgcggctagcctcggtatctcacgagcccacttctccgtcaccactccatgggccattgcttatatgggaccctcagctgacgccatgataaatggttcagatggtcgaaccacggttgaggatctcacgacaccgcccaagtggtttccctttccgaccaaagtatgctggcggaagcatgatcttgcccgactggtgccttacaaagctccggggatatctgatggataccgtatggggctggttcttaagggatctgattgtttgctttccaaatgttaccatgagtttggaactcaatggctacctcttttggagacactacaccaagtaccggtggttccggtgggattactgccaccggaaatacccggagacgagaaagatgaaacatgggtgtcaatcaagaaatggctcgatggtaaacaaaaaggcagtgtggtgtacgttgcattaggaagcgaggttttggtgagccaaaccgaggttgttgagttagcattgggtctcgagctttctgggttgccatttgtttgggcttatagaaaaccaaaaggtcccgcgaagtcagactcggtggagttgccagacgggttcgtggaacgaactcgtgaccgtgggttggtctggacgagttgggcacctcagttacgaatactgagccatgagtcggtttgtggtttcttgactcattgtggttctggatcaattgtggaagggctaatgtttggtcaccctctaatcatgctaccgatttttggggaccaacctctgaatgctcgattactggaggacaaacaggtgggaatcgagataccaagaaatgaggaagatggttgcttgaccaaggagtcggttgctagatcactgaggtccgttgttgtggaaaaagaaggggagatctacaaggcgaacgcgagggagctgagtaaaatctataacgacactaaggttgaaaaagaatatgtaagccaattcgtagactatttggaaaagaatgcgcgtgcggttgccatcgatcatgagagttaa

SEQ ID NO: 6 - protein, 485 aa, Stevia rebaudiana
MYNVTYHQNSKAMATSDSIVDDRKQLHVATFPWLAFGHILPYLQLSKLIAEKGHKVSFLSTTRNIQRLSSHISPLINVVQLTLPRVQELPEDAEATTDVHPEDIPYLKKASDGLQPEVTRFLEQHSPDWIIYDYTHYWLPSIAASLGISRAHFSVTTPWAIAYMGPSADAMINGSDGRTTVEDLTTPPKWFPFPTKVCWRKHDLARLVPYKAPGISDGYRMGLVLKGSDCLLSKCYHEFGTQWLPLLETLHQVPVVPVGLLPPEIPGDEKDETWVSIKKWLDGKQKGSVVYVALGSEVLVSQTEVVELALGLELSGLPFVWAYRKPKGPAKSDSVELPDGFVERTRDRGLVWTSWAPQLRILSHESVCGFLTHCGSGSIVEGLMFGHPLIMLPIFGDQPLNARLLEDKQVGIEIPRNEEDGCLTKESVARSLRSVVVEKEGEIYKANARELSKIYNDTKVEKEYVSQFVDYLEKNARAVAIDHES

SEQ ID NO: 7 - DNA, 1377 bp, Stevia rebaudiana
  CDS (1)..(1377)
atggaaaataaaacggagaccaccgttcgccggcgccggagaataatattattcccggtaccatttcaaggccacattaacccaattcttcagctagccaatgtgttgtactctaaaggattcagtatcaccatctttcacaccaacttcaacaaacccaaaacatctaattaccctcacttcactttcagattcatcctcgacaacgacccacaagacgaacgcatttccaatctaccgactcatggtccgctcgctggtatgcggattccgattatcaacgaacacggagctgacgaattacgacgcgaactggaactgttgatgttagcttctgaagaagatgaagaggtatcgtgtttaatcacggatgctctttggtacttcgcgcaatctgttgctgacagtcttaacctccgaccgcttgttttgatgacaagcagcttgtttaattttcatgcacatgtttcacttcctcagtttgatgagcttggttacctcgatcctgatgacaaaacccgtttggaagaacaagcgagtgggtttcctatgctaaaagtgaaagacatcaagtctgcgtattcgaactggcaaatactcaaagagatattagggaagatgataaaacaaacaaaagcatcttcaggagtcatctggaactcatttaaggaactcgaagagtctgagctcgaaactgttatccgtgagatcccggctccaagtttcttgataccactccccaagcatttgacagcctcttccagcagcttactagaccacgatcgaaccgtttttcaatggttagaccaacaaccgccaagttcggtactgtatgttagttttggtagtactagtgaagtggatgagaaagatttcttggaaatagctcgtgggttggttgatagcaagcagtcgtttttatgggtggttcgacctgggtttgtcaagggttcgacgtgggtcgaaccgttgccagatgggttcttgggtgaaagaggacgtattgtgaaatgggttccacagcaagaagtgctagctcatggagcaataggcgcattctggactcatagcggatggaactctacgttggaaagcgtttgtgaaggtgttcctatgattttctcggattttgggctcgatcaaccgttgaatgctagatacatgagtgatgttttgaaggtaggggtgtatttggaaaatgggtgggaaagaggagagatagcaaatgcaataagaagagttatggtggatgaagaaggagaatacattagacagaatgcaagagttttgaaacaaaaggcagatgtttctttgatgaagggtggttcgtcttacgaatcattagagtctctagtttcttacatttcatcgttgtaa

SEQ ID NO: 8 - protein, 458 aa, Stevia rebaudiana
MENKTETTVRRRRRIILFPVPFQGHINPILQLANVLYSKGFSITIFHTNFNKPKTSNYPHFTFRFILDNDPQDERISNLPTHGPLAGMRIPIINEHGADELRRELELLMLASEEDEEVSCLITDALWYFAQSVADSLNLRPLVLMTSSLFNFHAHVSLPQFDELGYLDPDDKTRLEEQASGFPMLKVKDIKSAYSNWQILKEILGKMIKQTKASSGVIWNSFKELEESELETVIREIPAPSFLIPLPKHLTASSSSLLDHDRTVFQWLDQQPPSSVLYVSFGSTSEVDEKDFLEIARGLVDSKQSFLWVVRPGFVKGSTWVEPLPDGFLGERGRIVKWVPQQEVLAHGAIGAFWTHSGWNSTLESVCEGVPMIFSDFGLDQPLNARYMSDVLKVGVYLENGWERGEIANAIRRVMVDEEGEYIRQNARVLKQKADVSLMKGGSSYESLESLVSYISSL

SEQ ID NO: 9 - DNA, 2004 bp, Arabidopsis thaliana
  CDS (1)..(2004)
atggatgatactacgtataagccaaagaacattctcattactggagctgctggatttattgcttctcatgttgccaacagattaatccgtaactatcctgattacaagatcgttgttcttgacaagcttgattactgttcagatctgaagaatcttgatccttctttttcttcaccaaatttcaagtttgtcaaaggagatatcgcgagtgatgatctcgttaactaccttctcatcactgaaaacattgatacgataatgcattttgctgctcaaactcatgttgataactcttttggtaatagctttgagtttaccaagaacaatatttatggtactcatgttcttttggaagcctgtaaagttacaggacagatcaggaggtttatccatgtgagtaccgatgaagtctatggagaaaccgatgaggatgctgctgtaggaaaccatgaagcttctcagctgttaccgacgaatccttactctgcaactaaggctggtgctgagatgcttgtgatggcttatggtagatcatatggattgcctgttattacgactcgcgggaacaatgtttatgggcctaaccagtttcctgaaaaaatgattcctaagttcatcttgttggctatgagtgggaagccgcttcccatccatggagatggatctaatgtccggagttacttgtactgcgaagacgttgctgaggcttttgaggttgttcttcacaaaggagaaatcggtcatgtctacaatgtcggcacaaaaagagaaaggagagtgatcgatgtggctagagacatctgcaaacttttcgggaaagaccctgagtcaagcattcagtttgtggagaaccggccctttaatgatcaaaggtacttccttgatgatcagaagctgaagaaattggggtggcaagagcgaacaaattgggaagatggattgaagaagacaatggactggtacactcagaatcctgagtggtggggtgatgtttctggagctttgcttcctcatccgagaatgcttatgatgcccggtggaagactttctgatggatctagtgagaagaaagacgtttcaagcaacacggtccagacatttacggttgtaacacctaagaatggtgattctggtgacaaagcttcgttgaagtttttgatctatggtaagactggttggcttggtggtcttctagggaaactatgtgagaagcaagggattacatatgagtatgggaaaggacgtctggaggatagagcttctcttgtggcggatattcgtagcatcaaacctactcatgtgtttaatgctgctggtttaactggcagacccaacgttgactggtgtgaatctcacaaaccagagaccattcgtgtaaatgtcgcaggtactttgactctagctgatgtttgcagagagaatgatctcttgatgatgaacttcgccaccggttgcatctttgagtatgacgctacacatcctgagggttcgggtataggtttcaaggaagaagacaagccaaatttctttggttctttctactcgaaaaccaaagccatggttgaggagctcttgagagaatttgacaatgtatgtaccttgagagtccggatgccaatctcctcagacctaaacaacccgagaaacttcatcacgaagatctcgcgctacaacaaagtggtggacatcccgaacagcatgaccgtactagacgagcttctcccaatctctatcgagatggcgaagagaaacctaagaggcatatggaatttcaccaacccaggggtggtgagccacaacgagatattggagatgtacaagaattacatcgagccaggttttaaatggtccaacttcacagtggaagaacaagcaaaggtcattgttgctgctcgaagcaacaacgaaatggatggatctaaactaagcaaggagttcccagagatgctctccatcaaagagtcactgctcaaatacgtctttgaaccaaacaagagaacctaa

SEQ ID NO: 10 - protein, 667 aa, Arabidopsis thaliana
MDDTTYKPKNILITGAAGFIASHVANRLIRNYPDYKIVVLDKLDYCSDLKNLDPSFSSPNFKFVKGDIASDDLVNYLLITENIDTIMHFAAQTHVDNSFGNSFEFTKNNIYGTHVLLEACKVTGQIRRFIHVSTDEVYGETDEDAAVGNHEASQLLPTNPYSATKAGAEMLVMAYGRSYGLPVITTRGNNVYGPNQFPEKMIPKFILLAMSGKPLPIHGDGSNVRSYLYCEDVAEAFEVVLHKGEIGHVYNVGTKRERRVIDVARDICKLFGKDPESSIQFVENRPFNDQRYFLDDQKLKKLGWQERTNWEDGLKKTMDWYTQNPEWWGDVSGALLPHPRMLMMPGGRLSDGSSEKKDVSSNTVQTFTVVTPKNGDSGDKASLKFLIYGKTGWLGGLLGKLCEKQGITYEYGKGRLEDRASLVADIRSIKPTHVFNAAGLTGRPNVDWCESHKPETIRVNVAGTLTLADVCRENDLLMMNFATGCIFEYDATHPEGSGIGFKEEDKPNFFGSFYSKTKAMVEELLREFDNVCTLRVRMPISSDLNNPRNFITKISRYNKVVDIPNSMTVLDELLPISIEMAKRNLRGIWNFTNPGVVSHNEILEMYKNYIEPGFKWSNFTVEEQAKVIVAARSNNEMDGSKLSKEFPEMLSIKESLLKYVFEPNKRT

SEQ ID NO: 11 - DNA, 60 bp, Stevia rebaudiana
gagtaaaatctataacgacactaaggtggaaaaagaatatgtaagccaattcgtagactt

SEQ ID NO: 12 - DNA, 33 bp, Artificial
  Artificial nucleic acid
cacccatatggatgcaatggctacaactgagaa

SEQ ID NO: 13 - DNA, 32 bp, Artificial
  Artificial nucleic acid
agatctctagtttcttgctagcacggtgattt

SEQ ID NO: 14 - DNA, 35 bp, Artificial
  Artificial nucleic acid
cacccatatggcggaacaacaaaagatcaagaaat

SEQ ID NO: 15 - DNA, 35 bp, Artificial
  Artificial nucleic acid
ggatccttaagccttaattagctcacttacaaatt

SEQ ID NO: 16 - DNA, 29 bp, Artificial
  Artificial nucleic acid
cacccatatggaaaataaaacggagacca

SEQ ID NO: 17 - DNA, 32 bp, Artificial
  Artificial nucleic acid
ggatccttacaacgatgaaatgtaagaaacta

SEQ ID NO: 18 - DNA, 33 bp, Artificial
  Artificial nucleic acid
acagatctatggatgcaatggctacaactgaga

SEQ ID NO: 19 - DNA, 34 bp, Artificial
  Artificial nucleic acid
tagtcgactagtttcttgctagcacggtgatttc

SEQ ID NO: 20 - DNA, 42 bp, Artificial
  Artificial nucleic acid
aagcggccgcatgtacaacgttacttatcatcaaaattcaaa

SEQ ID NO: 21 - DNA, 31 bp, Artificial
  Artificial nucleic acid
cgttaattaactctcatgatcgatggcaacc

SEQ ID NO: 22 - DNA, 34 bp, Artificial
  Artificial nucleic acid
aagcggccgcatggcggaacaacaaaagatcaag

SEQ ID NO: 23 - DNA, 37 bp, Artificial
  Artificial nucleic acid
cgttaattaagccttaattagctcacttacaaattcg

SEQ ID NO: 24 - DNA, 33 bp, Artificial
  Artificial nucleic acid
aaggatccatggaaaataaaacggagaccaccg

SEQ ID NO: 25 - DNA, 44 bp, Artificial
  Artificial nucleic acid
gcgtcgacttacaacgatgaaatgtaagaaactagagactctaa

SEQ ID NO: 26 - DNA, 33 bp, Artificial
  Artificial nucleic acid
ggatccatggatgatactacgtataagccaaag

SEQ ID NO: 27 - DNA, 32 bp, Artificial
  Artificial nucleic acid
ctcgagttaggttctcttgtttggttcaaaga

SEQ ID NO: 28 - DNA, 22 bp, Artificial
  Artificial nucleic acid
caagtccccaaccaaattccgt

SEQ ID NO: 29 - DNA, 21 bp, Artificial
  Artificial nucleic acid
cacgaacccgtctggcaactc

SEQ ID NO: 30 - DNA, 25 bp, Artificial
  Artificial nucleic acid
cccgtgtgatttcttccacttgttc

SEQ ID NO: 31 - DNA, 21 bp, Artificial
  Artificial nucleic acid
caagaacccatctggcaacgg

SEQ ID NO: 32 - DNA, 23 bp, Artificial
  Artificial nucleic acid
gctttgtcaccagaatcaccatt

SEQ ID NO: 33 - DNA, 28 bp, Artificial
  Artificial nucleic acid
gattattaaacttctttgcgtccatcca

SEQ ID NO: 34 - DNA, 32 bp, Artificial
  Artificial nucleic acid
cctctatactttaacgtcaaggagaaaaaacc

SEQ ID NO: 35 - DNA, 39 bp, Artificial
  Artificial nucleic acid
tgccgcgcggcagccatatgtacaacgttacttatcatc

SEQ ID NO: 36 - DNA, 39 bp, Artificial
  Artificial nucleic acid
gttagcagccggatccttaactctcatgatcgatggcaa